European Patent Specification EP 3 227 322 B1, published April 10, 2024. Title: CD44v6-derived cyclic peptides for treating metastasizing cancers. Applicant: Amcure GmbH. The sequence listing filed with the application follows.

SEQUENCE LISTING (40 sequences)

SEQ ID NO: 1 - protein, 5 aa, Artificial Sequence
  peptide
  VARIANT (1)..(1): /replace="Ala" /replace="Cys" /replace="Asp" /replace="Glu" /replace="Phe" /replace="Gly" /replace="His" /replace="Ile" /replace="Lys" /replace="Leu" /replace="Met" /replace="Pro" /replace="Gln" /replace="Arg" /replace="Ser" /replace="Thr" /replace="Val" /replace="Trp" /replace="Tyr"
  VARIANT (5)..(5): /replace="Ala" /replace="Cys" /replace="Asp" /replace="Phe" /replace="Gly" /replace="His" /replace="Ile" /replace="Lys" /replace="Leu" /replace="Met" /replace="Asn" /replace="Pro" /replace="Gln" /replace="Arg" /replace="Ser" /replace="Thr" /replace="Val" /replace="Trp" /replace="Tyr"
NRWHE

SEQ ID NO: 2 - protein, 5 aa, Artificial Sequence
  peptide
NRWHE

SEQ ID NO: 3 - protein, 5 aa, Artificial Sequence
  peptide
ARWHA

SEQ ID NO: 4 - protein, 5 aa, Artificial Sequence
  peptide
  VARIANT (1)..(1): /replace="Lys" /replace="Arg" /replace="Gln" /replace="Ala" /replace="Val" /replace="Leu" /replace="Ile"
  VARIANT (5)..(5): /replace="Asp" /replace="Ala" /replace="Val" /replace="Leu" /replace="Ile"
NRWHE

SEQ ID NO: 5 - protein, 5 aa, Artificial Sequence
  peptide
  VARIANT (1)..(1): /replace="Lys" /replace="Arg" /replace="Gln"
  VARIANT (5)..(5): /replace="Asp"
NRWHE

SEQ ID NO: 6 - protein, 14 aa, Artificial Sequence
  peptide
KEQWFGNRWHEGYR

SEQ ID NO: 7 - protein, 14 aa, Artificial Sequence
  peptide
  VARIANT (1)..(1): /replace="Ala" /replace="Cys" /replace="Asp" /replace="Glu" /replace="Phe" /replace="Gly" /replace="His" /replace="Ile" /replace="Leu" /replace="Met" /replace="Asn" /replace="Pro" /replace="Gln" /replace="Arg" /replace="Ser" /replace="Thr" /replace="Val" /replace="Trp" /replace="Tyr"
  VARIANT (2)..(2): /replace="Ala" /replace="Cys" /replace="Asp" /replace="Phe" /replace="Gly" /replace="His" /replace="Ile" /replace="Lys" /replace="Leu" /replace="Met" /replace="Asn" /replace="Pro" /replace="Gln" /replace="Arg" /replace="Ser" /replace="Thr" /replace="Val" /replace="Trp" /replace="Tyr"
  VARIANT (3)..(3): /replace="Ala" /replace="Cys" /replace="Asp" /replace="Glu" /replace="Phe" /replace="Gly" /replace="His" /replace="Ile" /replace="Lys" /replace="Leu" /replace="Met" /replace="Asn" /replace="Pro" /replace="Arg" /replace="Ser" /replace="Thr" /replace="Val" /replace="Trp" /replace="Tyr"
  VARIANT (4)..(4): /replace="Ala" /replace="Cys" /replace="Asp" /replace="Glu" /replace="Phe" /replace="Gly" /replace="His" /replace="Ile" /replace="Lys" /replace="Leu" /replace="Met" /replace="Asn" /replace="Pro" /replace="Gln" /replace="Arg" /replace="Ser" /replace="Thr" /replace="Val" /replace="Tyr"
  VARIANT (5)..(5): /replace="Ala" /replace="Cys" /replace="Asp" /replace="Glu" /replace="Gly" /replace="His" /replace="Ile" /replace="Lys" /replace="Leu" /replace="Met" /replace="Asn" /replace="Pro" /replace="Gln" /replace="Arg" /replace="Ser" /replace="Thr" /replace="Val" /replace="Trp" /replace="Tyr"
  VARIANT (6)..(6): /replace="Ala" /replace="Cys" /replace="Asp" /replace="Glu" /replace="Phe" /replace="His" /replace="Ile" /replace="Lys" /replace="Leu" /replace="Met" /replace="Asn" /replace="Pro" /replace="Gln" /replace="Arg" /replace="Ser" /replace="Thr" /replace="Val" /replace="Trp" /replace="Tyr"
  VARIANT (7)..(7): /replace="Ala" /replace="Cys" /replace="Asp" /replace="Glu" /replace="Phe" /replace="Gly" /replace="His" /replace="Ile" /replace="Lys" /replace="Leu" /replace="Met" /replace="Pro" /replace="Gln" /replace="Arg" /replace="Ser" /replace="Thr" /replace="Val" /replace="Trp" /replace="Tyr"
  VARIANT (11)..(11): /replace="Ala" /replace="Cys" /replace="Asp" /replace="Phe" /replace="Gly" /replace="His" /replace="Ile" /replace="Lys" /replace="Leu" /replace="Met" /replace="Asn" /replace="Pro" /replace="Gln" /replace="Arg" /replace="Ser" /replace="Thr" /replace="Val" /replace="Trp" /replace="Tyr"
  VARIANT (12)..(12): /replace="Ala" /replace="Cys" /replace="Asp" /replace="Glu" /replace="Phe" /replace="His" /replace="Ile" /replace="Lys" /replace="Leu" /replace="Met" /replace="Asn" /replace="Pro" /replace="Gln" /replace="Arg" /replace="Ser" /replace="Thr" /replace="Val" /replace="Trp" /replace="Tyr"
  VARIANT (13)..(13): /replace="Ala" /replace="Cys" /replace="Asp" /replace="Glu" /replace="Phe" /replace="Gly" /replace="His" /replace="Ile" /replace="Lys" /replace="Leu" /replace="Met" /replace="Asn" /replace="Pro" /replace="Gln" /replace="Arg" /replace="Ser" /replace="Thr" /replace="Val" /replace="Trp"
  VARIANT (14)..(14): /replace="Ala" /replace="Cys" /replace="Asp" /replace="Glu" /replace="Phe" /replace="Gly" /replace="His" /replace="Ile" /replace="Lys" /replace="Leu" /replace="Met" /replace="Asn" /replace="Pro" /replace="Gln" /replace="Ser" /replace="Thr" /replace="Val" /replace="Trp" /replace="Tyr"
KEQWFGNRWHEGYR

SEQ ID NO: 8 - protein, 14 aa, Artificial Sequence
  peptide
  VARIANT (1)..(1): /replace="Arg" /replace="Asn" /replace="Gln" /replace="Ala" /replace="Val" /replace="Leu" /replace="Ile"
  VARIANT (2)..(2): /replace="Asp" /replace="Ala" /replace="Val" /replace="Leu" /replace="Ile"
  VARIANT (3)..(3): /replace="Lys" /replace="Arg" /replace="Asn" /replace="Ala" /replace="Val" /replace="Leu" /replace="Ile"
  VARIANT (4)..(4): /replace="Phe" /replace="Tyr" /replace="Ala" /replace="Val" /replace="Leu" /replace="Ile"
  VARIANT (5)..(5): /replace="Trp" /replace="Tyr" /replace="Ala" /replace="Val" /replace="Leu" /replace="Ile"
  VARIANT (6)..(6): /replace="Ala" /replace="Val" /replace="Leu" /replace="Ile"
  VARIANT (7)..(7): /replace="Lys" /replace="Arg" /replace="Gln" /replace="Ala" /replace="Val" /replace="Leu" /replace="Ile"
  VARIANT (11)..(11): /replace="Asp" /replace="Ala" /replace="Val" /replace="Leu" /replace="Ile"
  VARIANT (12)..(12): /replace="Ala" /replace="Val" /replace="Leu" /replace="Ile"
  VARIANT (13)..(13): /replace="Phe" /replace="Trp" /replace="Ala" /replace="Val" /replace="Leu" /replace="Ile"
  VARIANT (14)..(14): /replace="Lys" /replace="Asn" /replace="Gln" /replace="Ala" /replace="Val" /replace="Leu" /replace="Ile"
KEQWFGNRWHEGYR

SEQ ID NO: 9 - protein, 14 aa, Artificial Sequence
  peptide
  VARIANT (1)..(1): /replace="Arg" /replace="Asn" /replace="Gln"
  VARIANT (2)..(2): /replace="Asp"
  VARIANT (3)..(3): /replace="Lys" /replace="Arg" /replace="Asn"
  VARIANT (4)..(4): /replace="Phe" /replace="Tyr"
  VARIANT (5)..(5): /replace="Trp" /replace="Tyr"
  VARIANT (6)..(6): /replace="Ala" /replace="Val" /replace="Leu" /replace="Ile"
  VARIANT (7)..(7): /replace="Lys" /replace="Arg" /replace="Gln"
  VARIANT (11)..(11): /replace="Asp"
  VARIANT (12)..(12): /replace="Ala" /replace="Val" /replace="Leu" /replace="Ile"
  VARIANT (13)..(13): /replace="Phe" /replace="Trp"
  VARIANT (14)..(14): /replace="Lys" /replace="Asn" /replace="Gln"
KEQWFGNRWHEGYR

SEQ ID NO: 10 - protein, 14 aa, Artificial Sequence
  peptide
KEKWFENEWQGKNP

SEQ ID NO: 11 - protein, 5 aa, Artificial Sequence
  peptide
NEWQG

SEQ ID NO: 12 - protein, 11 aa, Artificial Sequence
  peptide
WFENEWQGKNP

SEQ ID NO: 13 - protein, 11 aa, Artificial Sequence
  peptide
WFQNGWQGKNP

SEQ ID NO: 14 - protein, 11 aa, Artificial Sequence
  peptide
WFGNRWHEGYR

SEQ ID NO: 15 - protein, 5 aa, Artificial Sequence
  peptide
NAAAG

SEQ ID NO: 16 - protein, 8 aa, Artificial Sequence
  peptide
FGNRWHEG

SEQ ID NO: 17 - protein, 8 aa, Artificial Sequence
  peptide
  VARIANT (1)..(1): /replace="Ala" /replace="Cys" /replace="Asp" /replace="Glu" /replace="Gly" /replace="His" /replace="Ile" /replace="Lys" /replace="Leu" /replace="Met" /replace="Asn" /replace="Pro" /replace="Gln" /replace="Arg" /replace="Ser" /replace="Thr" /replace="Val" /replace="Trp" /replace="Tyr"
  VARIANT (2)..(2): /replace="Ala" /replace="Cys" /replace="Asp" /replace="Glu" /replace="Phe" /replace="His" /replace="Ile" /replace="Lys" /replace="Leu" /replace="Met" /replace="Asn" /replace="Pro" /replace="Gln" /replace="Arg" /replace="Ser" /replace="Thr" /replace="Val" /replace="Trp" /replace="Tyr"
  VARIANT (3)..(3): /replace="Ala" /replace="Cys" /replace="Asp" /replace="Glu" /replace="Phe" /replace="Gly" /replace="His" /replace="Ile" /replace="Lys" /replace="Leu" /replace="Met" /replace="Pro" /replace="Gln" /replace="Arg" /replace="Ser" /replace="Thr" /replace="Val" /replace="Trp" /replace="Tyr"
  VARIANT (7)..(7): /replace="Ala" /replace="Cys" /replace="Asp" /replace="Phe" /replace="Gly" /replace="His" /replace="Ile" /replace="Lys" /replace="Leu" /replace="Met" /replace="Asn" /replace="Pro" /replace="Gln" /replace="Arg" /replace="Ser" /replace="Thr" /replace="Val" /replace="Trp" /replace="Tyr"
  VARIANT (8)..(8): /replace="Ala" /replace="Cys" /replace="Asp" /replace="Glu" /replace="Phe" /replace="His" /replace="Ile" /replace="Lys" /replace="Leu" /replace="Met" /replace="Asn" /replace="Pro" /replace="Gln" /replace="Arg" /replace="Ser" /replace="Thr" /replace="Val" /replace="Trp" /replace="Tyr"
FGNRWHEG

SEQ ID NO: 18 - protein, 8 aa, Artificial Sequence
  peptide
KGNRWHEG

SEQ ID NO: 19 - protein, 14 aa, Artificial Sequence
  peptide
  VARIANT (1)..(1): /replace="Asn" /replace="Arg" /replace="Gln"
  VARIANT (2)..(2): /replace="Ala" /replace="Cys" /replace="Asp" /replace="Phe" /replace="Gly" /replace="His" /replace="Ile" /replace="Lys" /replace="Leu" /replace="Met" /replace="Asn" /replace="Pro" /replace="Gln" /replace="Arg" /replace="Ser" /replace="Thr" /replace="Val" /replace="Trp" /replace="Tyr"
  VARIANT (3)..(3): /replace="Ala" /replace="Cys" /replace="Asp" /replace="Glu" /replace="Phe" /replace="Gly" /replace="His" /replace="Ile" /replace="Lys" /replace="Leu" /replace="Met" /replace="Asn" /replace="Pro" /replace="Arg" /replace="Ser" /replace="Thr" /replace="Val" /replace="Trp" /replace="Tyr"
  VARIANT (4)..(4): /replace="Ala" /replace="Cys" /replace="Asp" /replace="Glu" /replace="Phe" /replace="Gly" /replace="His" /replace="Ile" /replace="Lys" /replace="Leu" /replace="Met" /replace="Asn" /replace="Pro" /replace="Gln" /replace="Arg" /replace="Ser" /replace="Thr" /replace="Val" /replace="Tyr"
  VARIANT (5)..(5): /replace="Ala" /replace="Cys" /replace="Asp" /replace="Glu" /replace="Gly" /replace="His" /replace="Ile" /replace="Lys" /replace="Leu" /replace="Met" /replace="Asn" /replace="Pro" /replace="Gln" /replace="Arg" /replace="Ser" /replace="Thr" /replace="Val" /replace="Trp" /replace="Tyr"
  VARIANT (6)..(6): /replace="Ala" /replace="Cys" /replace="Asp" /replace="Glu" /replace="Phe" /replace="His" /replace="Ile" /replace="Lys" /replace="Leu" /replace="Met" /replace="Asn" /replace="Pro" /replace="Gln" /replace="Arg" /replace="Ser" /replace="Thr" /replace="Val" /replace="Trp" /replace="Tyr"
  VARIANT (7)..(7): /replace="Ala" /replace="Cys" /replace="Asp" /replace="Glu" /replace="Phe" /replace="Gly" /replace="His" /replace="Ile" /replace="Lys" /replace="Leu" /replace="Met" /replace="Pro" /replace="Gln" /replace="Arg" /replace="Ser" /replace="Thr" /replace="Val" /replace="Trp" /replace="Tyr"
  VARIANT (11)..(11): /replace="Ala" /replace="Cys" /replace="Asp" /replace="Phe" /replace="Gly" /replace="His" /replace="Ile" /replace="Lys" /replace="Leu" /replace="Met" /replace="Asn" /replace="Pro" /replace="Gln" /replace="Arg" /replace="Ser" /replace="Thr" /replace="Val" /replace="Trp" /replace="Tyr"
  VARIANT (12)..(12): /replace="Ala" /replace="Cys" /replace="Asp" /replace="Glu" /replace="Phe" /replace="His" /replace="Ile" /replace="Lys" /replace="Leu" /replace="Met" /replace="Asn" /replace="Pro" /replace="Gln" /replace="Arg" /replace="Ser" /replace="Thr" /replace="Val" /replace="Trp" /replace="Tyr"
  VARIANT (13)..(13): /replace="Ala" /replace="Cys" /replace="Asp" /replace="Glu" /replace="Phe" /replace="Gly" /replace="His" /replace="Ile" /replace="Lys" /replace="Leu" /replace="Met" /replace="Asn" /replace="Pro" /replace="Gln" /replace="Arg" /replace="Ser" /replace="Thr" /replace="Val" /replace="Trp"
  VARIANT (14)..(14): /replace="Ala" /replace="Cys" /replace="Asp" /replace="Glu" /replace="Phe" /replace="Gly" /replace="His" /replace="Ile" /replace="Lys" /replace="Leu" /replace="Met" /replace="Asn" /replace="Pro" /replace="Gln" /replace="Ser" /replace="Thr" /replace="Val" /replace="Trp" /replace="Tyr"
KEQWFGNRWHEGYR

SEQ ID NO: 20 - protein, 14 aa, Artificial Sequence
  peptide
  VARIANT (1)..(1): /replace="Asn" /replace="Gln" /replace="Arg"
  VARIANT (2)..(2): /replace="Asp"
  VARIANT (3)..(3): /replace="Lys" /replace="Asn" /replace="Arg" /replace="Ala" /replace="Val" /replace="Leu" /replace="Ile"
  VARIANT (4)..(4): /replace="Ala" /replace="Phe" /replace="Ile" /replace="Leu" /replace="Val" /replace="Tyr"
  VARIANT (5)..(5): /replace="Ala" /replace="Ile" /replace="Leu" /replace="Val" /replace="Trp" /replace="Tyr"
  VARIANT (6)..(6): /replace="Ala" /replace="Ile" /replace="Leu" /replace="Val"
  VARIANT (7)..(7): /replace="Gln" /replace="Arg" /replace="Lys"
  VARIANT (11)..(11): /replace="Asp"
  VARIANT (12)..(12): /replace="Ala" /replace="Ile" /replace="Leu" /replace="Val"
  VARIANT (13)..(13): /replace="Ala" /replace="Phe" /replace="Ile" /replace="Leu" /replace="Val" /replace="Trp"
  VARIANT (14)..(14): /replace="Lys" /replace="Gln" /replace="Asn"
KEQWFGNRWHEGYR

SEQ ID NO: 21 - protein, 13 aa, Artificial Sequence
  peptide
  VARIANT (1)..(1): /replace="Ala" /replace="Cys" /replace="Asp" /replace="Glu" /replace="Phe" /replace="Gly" /replace="His" /replace="Ile" /replace="Leu" /replace="Met" /replace="Asn" /replace="Pro" /replace="Gln" /replace="Arg" /replace="Ser" /replace="Thr" /replace="Val" /replace="Trp" /replace="Tyr"
  VARIANT (2)..(2): /replace="Ala" /replace="Cys" /replace="Asp" /replace="Glu" /replace="Phe" /replace="Gly" /replace="His" /replace="Ile" /replace="Lys" /replace="Leu" /replace="Met" /replace="Asn" /replace="Pro" /replace="Arg" /replace="Ser" /replace="Thr" /replace="Val" /replace="Trp" /replace="Tyr"
  VARIANT (3)..(3): /replace="Ala" /replace="Cys" /replace="Asp" /replace="Glu" /replace="Phe" /replace="Gly" /replace="His" /replace="Ile" /replace="Lys" /replace="Leu" /replace="Met" /replace="Asn" /replace="Pro" /replace="Gln" /replace="Arg" /replace="Ser" /replace="Thr" /replace="Val" /replace="Tyr"
  VARIANT (4)..(4): /replace="Ala" /replace="Cys" /replace="Asp" /replace="Glu" /replace="Gly" /replace="His" /replace="Ile" /replace="Lys" /replace="Leu" /replace="Met" /replace="Asn" /replace="Pro" /replace="Gln" /replace="Arg" /replace="Ser" /replace="Thr" /replace="Val" /replace="Trp" /replace="Tyr"
  VARIANT (5)..(5): /replace="Ala" /replace="Cys" /replace="Asp" /replace="Glu" /replace="Phe" /replace="His" /replace="Ile" /replace="Lys" /replace="Leu" /replace="Met" /replace="Asn" /replace="Pro" /replace="Gln" /replace="Arg" /replace="Ser" /replace="Thr" /replace="Val" /replace="Trp" /replace="Tyr"
  VARIANT (6)..(6): /replace="Ala" /replace="Cys" /replace="Asp" /replace="Glu" /replace="Phe" /replace="Gly" /replace="His" /replace="Ile" /replace="Lys" /replace="Leu" /replace="Met" /replace="Pro" /replace="Gln" /replace="Arg" /replace="Ser" /replace="Thr" /replace="Val" /replace="Trp" /replace="Tyr"
  VARIANT (10)..(10): /replace="Ala" /replace="Cys" /replace="Asp" /replace="Phe" /replace="Gly" /replace="His" /replace="Ile" /replace="Lys" /replace="Leu" /replace="Met" /replace="Asn" /replace="Pro" /replace="Gln" /replace="Arg" /replace="Ser" /replace="Thr" /replace="Val" /replace="Trp" /replace="Tyr"
  VARIANT (11)..(11): /replace="Ala" /replace="Cys" /replace="Asp" /replace="Glu" /replace="Phe" /replace="His" /replace="Ile" /replace="Lys" /replace="Leu" /replace="Met" /replace="Asn" /replace="Pro" /replace="Gln" /replace="Arg" /replace="Ser" /replace="Thr" /replace="Val" /replace="Trp" /replace="Tyr"
  VARIANT (12)..(12): /replace="Ala" /replace="Cys" /replace="Asp" /replace="Glu" /replace="Phe" /replace="Gly" /replace="His" /replace="Ile" /replace="Lys" /replace="Leu" /replace="Met" /replace="Asn" /replace="Pro" /replace="Gln" /replace="Arg" /replace="Ser" /replace="Thr" /replace="Val" /replace="Trp"
  VARIANT (13)..(13): /replace="Ala" /replace="Cys" /replace="Asp" /replace="Glu" /replace="Phe" /replace="Gly" /replace="His" /replace="Ile" /replace="Lys" /replace="Leu" /replace="Met" /replace="Asn" /replace="Pro" /replace="Gln" /replace="Ser" /replace="Thr" /replace="Val" /replace="Trp" /replace="Tyr"
KQWFGNRWHEGYR

SEQ ID NO: 22 - protein, 12 aa, Artificial Sequence
  peptide
  VARIANT (1)..(1): /replace="Ala" /replace="Cys" /replace="Asp" /replace="Glu" /replace="Phe" /replace="Gly" /replace="His" /replace="Ile" /replace="Leu" /replace="Met" /replace="Asn" /replace="Pro" /replace="Gln" /replace="Arg" /replace="Ser" /replace="Thr" /replace="Val" /replace="Trp" /replace="Tyr"
  VARIANT (2)..(2): /replace="Ala" /replace="Cys" /replace="Asp" /replace="Glu" /replace="Phe" /replace="Gly" /replace="His" /replace="Ile" /replace="Lys" /replace="Leu" /replace="Met" /replace="Asn" /replace="Pro" /replace="Arg" /replace="Ser" /replace="Thr" /replace="Val" /replace="Gln" /replace="Tyr"
  VARIANT (3)..(3): /replace="Ala" /replace="Cys" /replace="Asp" /replace="Glu" /replace="Trp" /replace="Gly" /replace="His" /replace="Ile" /replace="Lys" /replace="Leu" /replace="Met" /replace="Asn" /replace="Pro" /replace="Gln" /replace="Arg" /replace="Ser" /replace="Thr" /replace="Val" /replace="Tyr"
  VARIANT (4)..(4): /replace="Ala" /replace="Cys" /replace="Asp" /replace="Glu" /replace="Phe" /replace="His" /replace="Ile" /replace="Lys" /replace="Leu" /replace="Met" /replace="Asn" /replace="Pro" /replace="Gln" /replace="Arg" /replace="Ser" /replace="Thr" /replace="Val" /replace="Trp" /replace="Tyr"
  VARIANT (5)..(5): /replace="Ala" /replace="Cys" /replace="Asp" /replace="Glu" /replace="Phe" /replace="His" /replace="Ile" /replace="Lys" /replace="Leu" /replace="Met" /replace="Gly" /replace="Pro" /replace="Gln" /replace="Arg" /replace="Ser" /replace="Thr" /replace="Val" /replace="Trp" /replace="Tyr"
  VARIANT (9)..(9): /replace="Ala" /replace="Cys" /replace="Asp" /replace="Gly" /replace="Phe" /replace="His" /replace="Ile" /replace="Lys" /replace="Leu" /replace="Met" /replace="Asn" /replace="Pro" /replace="Gln" /replace="Arg" /replace="Ser" /replace="Thr" /replace="Val" /replace="Trp" /replace="Tyr"
  VARIANT (10)..(10): /replace="Ala" /replace="Cys" /replace="Asp" /replace="Glu" /replace="Phe" /replace="Tyr" /replace="His" /replace="Ile" /replace="Lys" /replace="Leu" /replace="Met" /replace="Asn" /replace="Pro" /replace="Gln" /replace="Arg" /replace="Ser" /replace="Thr" /replace="Val" /replace="Trp"
  VARIANT (11)..(11): /replace="Ala" /replace="Cys" /replace="Asp" /replace="Glu" /replace="Phe" /replace="Gly" /replace="His" /replace="Ile" /replace="Lys" /replace="Leu" /replace="Met" /replace="Asn" /replace="Pro" /replace="Gln" /replace="Ser" /replace="Thr" /replace="Val" /replace="Trp" /replace="Tyr"
KWFGNRWHEGYR

SEQ ID NO: 23 - protein, 11 aa, Artificial Sequence
  peptide
  VARIANT (1)..(1): /replace="Ala" /replace="Cys" /replace="Asp" /replace="Glu" /replace="Phe" /replace="Gly" /replace="His" /replace="Ile" /replace="Leu" /replace="Met" /replace="Asn" /replace="Pro" /replace="Gln" /replace="Arg" /replace="Ser" /replace="Thr" /replace="Val" /replace="Trp" /replace="Tyr"
  VARIANT (2)..(2): /replace="Ala" /replace="Cys" /replace="Asp" /replace="Glu" /replace="Gln" /replace="Gly" /replace="His" /replace="Ile" /replace="Lys" /replace="Leu" /replace="Met" /replace="Asn" /replace="Pro" /replace="Arg" /replace="Ser" /replace="Thr" /replace="Val" /replace="Trp" /replace="Tyr"
  VARIANT (3)..(3): /replace="Ala" /replace="Cys" /replace="Asp" /replace="Glu" /replace="Phe" /replace="Trp" /replace="His" /replace="Ile" /replace="Lys" /replace="Leu" /replace="Met" /replace="Asn" /replace="Pro" /replace="Gln" /replace="Arg" /replace="Ser" /replace="Thr" /replace="Val" /replace="Tyr"
  VARIANT (4)..(4): /replace="Ala" /replace="Cys" /replace="Asp" /replace="Glu" /replace="Gly" /replace="His" /replace="Ile" /replace="Lys" /replace="Leu" /replace="Met" /replace="Phe" /replace="Pro" /replace="Gln" /replace="Arg" /replace="Ser" /replace="Thr" /replace="Val" /replace="Trp" /replace="Tyr"
  VARIANT (8)..(8): /replace="Ala" /replace="Cys" /replace="Asp" /replace="Gly" /replace="Phe" /replace="His" /replace="Ile" /replace="Lys" /replace="Leu" /replace="Met" /replace="Asn" /replace="Pro" /replace="Gln" /replace="Arg" /replace="Ser" /replace="Thr" /replace="Val" /replace="Trp" /replace="Tyr"
  VARIANT (9)..(9): /replace="Ala" /replace="Cys" /replace="Asp" /replace="Glu" /replace="Phe" /replace="Asn" /replace="His" /replace="Ile" /replace="Lys" /replace="Leu" /replace="Met" /replace="Pro" /replace="Gln" /replace="Arg" /replace="Ser" /replace="Thr" /replace="Val" /replace="Trp" /replace="Tyr"
  VARIANT (10)..(10): /replace="Ala" /replace="Cys" /replace="Asp" /replace="Phe" /replace="Gly" /replace="His" /replace="Ile" /replace="Lys" /replace="Leu" /replace="Met" /replace="Asn" /replace="Pro" /replace="Gln" /replace="Arg" /replace="Ser" /replace="Thr" /replace="Val" /replace="Trp" /replace="Glu"
  VARIANT (11)..(11): /replace="Ala" /replace="Cys" /replace="Asp" /replace="Glu" /replace="Phe" /replace="His" /replace="Ile" /replace="Lys" /replace="Leu" /replace="Met" /replace="Asn" /replace="Pro" /replace="Gln" /replace="Gly" /replace="Ser" /replace="Thr" /replace="Val" /replace="Trp" /replace="Tyr"
KFGNRWHEGYR

SEQ ID NO: 24 - protein, 10 aa, Artificial Sequence
  peptide
  VARIANT (1)..(1): /replace="Ala" /replace="Cys" /replace="Asp" /replace="Glu" /replace="Phe" /replace="Gly" /replace="His" /replace="Ile" /replace="Leu" /replace="Met" /replace="Asn" /replace="Pro" /replace="Gln" /replace="Arg" /replace="Ser" /replace="Thr" /replace="Val" /replace="Trp" /replace="Tyr"
  VARIANT (2)..(2): /replace="Ala" /replace="Cys" /replace="Asp" /replace="Glu" /replace="Phe" /replace="Gln" /replace="His" /replace="Ile" /replace="Lys" /replace="Leu" /replace="Met" /replace="Asn" /replace="Pro" /replace="Arg" /replace="Ser" /replace="Thr" /replace="Val" /replace="Trp" /replace="Tyr"
  VARIANT (3)..(3): /replace="Ala" /replace="Cys" /replace="Asp" /replace="Glu" /replace="Phe" /replace="Gly" /replace="His" /replace="Ile" /replace="Lys" /replace="Leu" /replace="Met" /replace="Trp" /replace="Pro" /replace="Gln" /replace="Arg" /replace="Ser" /replace="Thr" /replace="Val" /replace="Tyr"
  VARIANT (7)..(7): /replace="Ala" /replace="Cys" /replace="Asp" /replace="Phe" /replace="Gly" /replace="His" /replace="Ile" /replace="Lys" /replace="Leu" /replace="Met" /replace="Asn" /replace="Pro" /replace="Gln" /replace="Arg" /replace="Ser" /replace="Thr" /replace="Val" /replace="Trp" /replace="Tyr"
  VARIANT (8)..(8): /replace="Ala" /replace="Cys" /replace="Asp" /replace="Glu" /replace="Phe" /replace="His" /replace="Ile" /replace="Lys" /replace="Leu" /replace="Met" /replace="Asn" /replace="Pro" /replace="Gln" /replace="Arg" /replace="Ser" /replace="Thr" /replace="Val" /replace="Trp" /replace="Tyr"
  VARIANT (9)..(9): /replace="Ala" /replace="Cys" /replace="Asp" /replace="Glu" /replace="Phe" /replace="Gly" /replace="His" /replace="Ile" /replace="Lys" /replace="Leu" /replace="Met" /replace="Pro" /replace="Gln" /replace="Arg" /replace="Ser" /replace="Thr" /replace="Val" /replace="Trp" /replace="Asn"
  VARIANT (10)..(10): /replace="Ala" /replace="Cys" /replace="Asp" /replace="Phe" /replace="Gly" /replace="His" /replace="Ile" /replace="Lys" /replace="Leu" /replace="Met" /replace="Asn" /replace="Pro" /replace="Gln" /replace="Glu" /replace="Ser" /replace="Thr" /replace="Val" /replace="Trp" /replace="Tyr"
KGNRWHEGYR

SEQ ID NO: 25 - protein, 9 aa, Artificial Sequence
  peptide
  VARIANT (1)..(1): /replace="Ala" /replace="Cys" /replace="Asp" /replace="Glu" /replace="Phe" /replace="Gly" /replace="His" /replace="Ile" /replace="Leu" /replace="Met" /replace="Asn" /replace="Pro" /replace="Gln" /replace="Arg" /replace="Ser" /replace="Thr" /replace="Val" /replace="Trp" /replace="Tyr"
  VARIANT (2)..(2): /replace="Ala" /replace="Cys" /replace="Asp" /replace="Glu" /replace="Phe" /replace="Gly" /replace="His" /replace="Ile" /replace="Lys" /replace="Leu" /replace="Met" /replace="Gln" /replace="Pro" /replace="Arg" /replace="Ser" /replace="Thr" /replace="Val" /replace="Trp" /replace="Tyr"
  VARIANT (6)..(6): /replace="Ala" /replace="Cys" /replace="Asp" /replace="Trp" /replace="Phe" /replace="Gly" /replace="His" /replace="Ile" /replace="Lys" /replace="Leu" /replace="Met" /replace="Asn" /replace="Pro" /replace="Gln" /replace="Arg" /replace="Ser" /replace="Thr" /replace="Val" /replace="Tyr"
  VARIANT (7)..(7): /replace="Ala" /replace="Cys" /replace="Asp" /replace="Glu" /replace="Phe" /replace="His" /replace="Ile" /replace="Lys" /replace="Leu" /replace="Met" /replace="Asn" /replace="Pro" /replace="Gln" /replace="Arg" /replace="Ser" /replace="Thr" /replace="Val" /replace="Trp" /replace="Tyr"
  VARIANT (8)..(8): /replace="Ala" /replace="Cys" /replace="Asp" /replace="Glu" /replace="Phe" /replace="His" /replace="Ile" /replace="Lys" /replace="Leu" /replace="Met" /replace="Asn" /replace="Pro" /replace="Gln" /replace="Arg" /replace="Ser" /replace="Thr" /replace="Val" /replace="Trp" /replace="Gly"
  VARIANT (9)..(9): /replace="Ala" /replace="Cys" /replace="Asp" /replace="Glu" /replace="Phe" /replace="Gly" /replace="His" /replace="Ile" /replace="Lys" /replace="Leu" /replace="Met" /replace="Pro" /replace="Gln" /replace="Asn" /replace="Ser" /replace="Thr" /replace="Val" /replace="Trp" /replace="Tyr"
KNRWHEGYR

SEQ ID NO: 26 - protein, 8 aa, Artificial Sequence
  peptide
  VARIANT (1)..(1): /replace="Ala" /replace="Cys" /replace="Asp" /replace="Glu" /replace="Phe" /replace="Gly" /replace="His" /replace="Ile" /replace="Leu" /replace="Met" /replace="Asn" /replace="Pro" /replace="Gln" /replace="Arg" /replace="Ser" /replace="Thr" /replace="Val" /replace="Trp" /replace="Tyr"
  VARIANT (5)..(5): /replace="Ala" /replace="Cys" /replace="Asp" /replace="Gln" /replace="Phe" /replace="Gly" /replace="His" /replace="Ile" /replace="Lys" /replace="Leu" /replace="Met" /replace="Asn" /replace="Pro" /replace="Arg" /replace="Ser" /replace="Thr" /replace="Val" /replace="Trp" /replace="Tyr"
  VARIANT (6)..(6): /replace="Ala" /replace="Cys" /replace="Asp" /replace="Glu" /replace="Phe" /replace="Trp" /replace="His" /replace="Ile" /replace="Lys" /replace="Leu" /replace="Met" /replace="Asn" /replace="Pro" /replace="Gln" /replace="Arg" /replace="Ser" /replace="Thr" /replace="Val" /replace="Tyr"
  VARIANT (7)..(7): /replace="Ala" /replace="Cys" /replace="Asp" /replace="Glu" /replace="Gly" /replace="His" /replace="Ile" /replace="Lys" /replace="Leu" /replace="Met" /replace="Asn" /replace="Pro" /replace="Gln" /replace="Arg" /replace="Ser" /replace="Thr" /replace="Val" /replace="Trp" /replace="Phe"
  VARIANT (8)..(8): /replace="Ala" /replace="Cys" /replace="Asp" /replace="Glu" /replace="Phe" /replace="His" /replace="Ile" /replace="Lys" /replace="Leu" /replace="Met" /replace="Asn" /replace="Pro" /replace="Gln" /replace="Gly" /replace="Ser" /replace="Thr" /replace="Val" /replace="Trp" /replace="Tyr"
KRWHEGYR

SEQ ID NO: 27 - protein, 11 aa, Artificial Sequence
  peptide
  VARIANT (1)..(1): /replace="Asn" /replace="Gln" /replace="Arg"
  VARIANT (2)..(2): /replace="Asp"
  VARIANT (3)..(3): /replace="Lys" /replace="Asn" /replace="Arg" /replace="Ala" /replace="Val" /replace="Leu" /replace="Ile"
  VARIANT (4)..(4): /replace="Ala" /replace="Phe" /replace="Ile" /replace="Leu" /replace="Val" /replace="Tyr"
  VARIANT (5)..(5): /replace="Ala" /replace="Ile" /replace="Leu" /replace="Val" /replace="Trp" /replace="Tyr"
  VARIANT (6)..(6): /replace="Ala" /replace="Ile" /replace="Leu" /replace="Val"
  VARIANT (7)..(7): /replace="Gln" /replace="Arg" /replace="Lys"
  VARIANT (11)..(11): /replace="Asp"
  VARIANT (12)..(12): /replace="Ala" /replace="Ile" /replace="Leu" /replace="Val"
  VARIANT (13)..(13): /replace="Ala" /replace="Phe" /replace="Ile" /replace="Leu" /replace="Val" /replace="Trp"
  VARIANT (14)..(14): /replace="Lys" /replace="Gln" /replace="Asn"
KEQWFGNRWHE

SEQ ID NO: 28 - protein, 10 aa, Artificial Sequence
  peptide
  VARIANT (1)..(1): /replace="Asn" /replace="Gln" /replace="Arg"
  VARIANT (2)..(2): /replace="Ala" /replace="Cys" /replace="Asp" /replace="Glu" /replace="Phe" /replace="Gly" /replace="His" /replace="Ile" /replace="Lys" /replace="Leu" /replace="Met" /replace="Asn" /replace="Pro" /replace="Arg" /replace="Ser" /replace="Thr" /replace="Val" /replace="Trp" /replace="Tyr"
  VARIANT (3)..(3): /replace="Ala" /replace="Cys" /replace="Asp" /replace="Glu" /replace="Phe" /replace="Gly" /replace="His" /replace="Ile" /replace="Lys" /replace="Leu" /replace="Met" /replace="Asn" /replace="Pro" /replace="Gln" /replace="Arg" /replace="Ser" /replace="Thr" /replace="Val" /replace="Tyr"
  VARIANT (4)..(4): /replace="Ala" /replace="Cys" /replace="Asp" /replace="Glu" /replace="Gly" /replace="His" /replace="Ile" /replace="Lys" /replace="Leu" /replace="Met" /replace="Asn" /replace="Pro" /replace="Gln" /replace="Arg" /replace="Ser" /replace="Thr" /replace="Val" /replace="Trp" /replace="Tyr"
  VARIANT (5)..(5): /replace="Ala" /replace="Cys" /replace="Asp" /replace="Glu" /replace="Phe" /replace="His" /replace="Ile" /replace="Lys" /replace="Leu" /replace="Met" /replace="Asn" /replace="Pro" /replace="Gln" /replace="Arg" /replace="Ser" /replace="Thr" /replace="Val" /replace="Trp" /replace="Tyr"
  VARIANT (6)..(6): /replace="Ala" /replace="Cys" /replace="Asp" /replace="Glu" /replace="Phe" /replace="Gly" /replace="His" /replace="Ile" /replace="Lys" /replace="Leu" /replace="Met" /replace="Pro" /replace="Gln" /replace="Arg" /replace="Ser" /replace="Thr" /replace="Val" /replace="Trp" /replace="Tyr"
  VARIANT (10)..(10): /replace="Ala" /replace="Cys" /replace="Asp" /replace="Phe" /replace="Gly" /replace="His" /replace="Ile" /replace="Lys" /replace="Leu" /replace="Met" /replace="Asn" /replace="Pro" /replace="Gln" /replace="Arg" /replace="Ser" /replace="Thr" /replace="Val" /replace="Trp" /replace="Tyr"
KQWFGNRWHE

SEQ ID NO: 29 - protein, 9 aa, Artificial Sequence
  peptide
  VARIANT (1)..(1): /replace="Asn" /replace="Gln" /replace="Arg"
  VARIANT (2)..(2): /replace="Ala" /replace="Cys" /replace="Asp" /replace="Glu" /replace="Phe" /replace="Gly" /replace="His" /replace="Ile" /replace="Lys" /replace="Leu" /replace="Met" /replace="Asn" /replace="Pro" /replace="Arg" /replace="Ser" /replace="Thr" /replace="Val" /replace="Gln" /replace="Tyr"
  VARIANT (3)..(3): /replace="Ala" /replace="Cys" /replace="Asp" /replace="Glu" /replace="Trp" /replace="Gly" /replace="His" /replace="Ile" /replace="Lys" /replace="Leu" /replace="Met" /replace="Asn" /replace="Pro" /replace="Gln" /replace="Arg" /replace="Ser" /replace="Thr" /replace="Val" /replace="Tyr"
  VARIANT (4)..(4): /replace="Ala" /replace="Cys" /replace="Asp" /replace="Glu" /replace="Phe" /replace="His" /replace="Ile" /replace="Lys" /replace="Leu" /replace="Met" /replace="Asn" /replace="Pro" /replace="Gln" /replace="Arg" /replace="Ser" /replace="Thr" /replace="Val" /replace="Trp" /replace="Tyr"
  VARIANT (5)..(5): /replace="Ala" /replace="Cys" /replace="Asp" /replace="Glu" /replace="Phe" /replace="His" /replace="Ile" /replace="Lys" /replace="Leu" /replace="Met" /replace="Gly" /replace="Pro" /replace="Gln" /replace="Arg" /replace="Ser" /replace="Thr" /replace="Val" /replace="Trp" /replace="Tyr"
  VARIANT (9)..(9): /replace="Ala" /replace="Cys" /replace="Asp" /replace="Gly" /replace="Phe" /replace="His" /replace="Ile" /replace="Lys" /replace="Leu" /replace="Met" /replace="Asn" /replace="Pro" /replace="Gln" /replace="Arg" /replace="Ser" /replace="Thr" /replace="Val" /replace="Trp" /replace="Tyr"
KWFGNRWHE

SEQ ID NO: 30 - protein, 8 aa, Artificial Sequence
  peptide
  VARIANT (1)..(1): /replace="Asn" /replace="Gln" /replace="Arg"
  VARIANT (2)..(2): /replace="Ala" /replace="Cys" /replace="Asp" /replace="Glu" /replace="Gln" /replace="Gly" /replace="His" /replace="Ile" /replace="Lys" /replace="Leu" /replace="Met" /replace="Asn" /replace="Pro" /replace="Arg" /replace="Ser" /replace="Thr" /replace="Val" /replace="Trp" /replace="Tyr"
  VARIANT (3)..(3): /replace="Ala" /replace="Cys" /replace="Asp" /replace="Glu" /replace="Phe" /replace="Trp" /replace="His" /replace="Ile" /replace="Lys" /replace="Leu" /replace="Met" /replace="Asn" /replace="Pro" /replace="Gln" /replace="Arg" /replace="Ser" /replace="Thr" /replace="Val" /replace="Tyr"
  VARIANT (4)..(4): /replace="Ala" /replace="Cys" /replace="Asp" /replace="Glu" /replace="Gly" /replace="His" /replace="Ile" /replace="Lys" /replace="Leu" /replace="Met" /replace="Phe" /replace="Pro" /replace="Gln" /replace="Arg" /replace="Ser" /replace="Thr" /replace="Val" /replace="Trp" /replace="Tyr"
  VARIANT (8)..(8): /replace="Ala" /replace="Cys" /replace="Asp" /replace="Gly" /replace="Phe" /replace="His" /replace="Ile" /replace="Lys" /replace="Leu" /replace="Met" /replace="Asn" /replace="Pro" /replace="Gln" /replace="Arg" /replace="Ser" /replace="Thr" /replace="Val" /replace="Trp" /replace="Tyr"
KFGNRWHE

SEQ ID NO: 31 - protein, 7 aa, Artificial Sequence
  peptide
  VARIANT (1)..(1): /replace="Ala" /replace="Cys" /replace="Asp" /replace="Glu" /replace="Phe" /replace="Gly" /replace="His" /replace="Ile" /replace="Leu" /replace="Met" /replace="Asn" /replace="Pro" /replace="Gln" /replace="Arg" /replace="Ser" /replace="Thr" /replace="Val" /replace="Trp" /replace="Tyr"
  VARIANT (2)..(2): /replace="Ala" /replace="Cys" /replace="Asp" /replace="Glu" /replace="Phe" /replace="Gln" /replace="His" /replace="Ile" /replace="Lys" /replace="Leu" /replace="Met" /replace="Asn" /replace="Pro" /replace="Arg" /replace="Ser" /replace="Thr" /replace="Val" /replace="Trp" /replace="Tyr"
  VARIANT (3)..(3): /replace="Ala" /replace="Cys" /replace="Asp" /replace="Glu" /replace="Phe" /replace="Gly" /replace="His" /replace="Ile" /replace="Lys" /replace="Leu" /replace="Met" /replace="Trp" /replace="Pro" /replace="Gln" /replace="Arg" /replace="Ser" /replace="Thr" /replace="Val" /replace="Tyr"
  VARIANT (7)..(7): /replace="Ala" /replace="Cys" /replace="Asp" /replace="Phe" /replace="Gly" /replace="His" /replace="Ile" /replace="Lys" /replace="Leu" /replace="Met" /replace="Asn" /replace="Pro" /replace="Gln" /replace="Arg" /replace="Ser" /replace="Thr" /replace="Val" /replace="Trp" /replace="Tyr"
KGNRWHE

SEQ ID NO: 32 - protein, 6 aa, Artificial Sequence
  peptide
  VARIANT (1)..(1): /replace="Ala" /replace="Cys" /replace="Asp" /replace="Glu" /replace="Phe" /replace="Gly" /replace="His" /replace="Ile" /replace="Leu" /replace="Met" /replace="Asn" /replace="Pro" /replace="Gln" /replace="Arg" /replace="Ser" /replace="Thr" /replace="Val" /replace="Trp" /replace="Tyr"
  VARIANT (2)..(2): /replace="Ala" /replace="Cys" /replace="Asp" /replace="Glu" /replace="Phe" /replace="Gly" /replace="His" /replace="Ile" /replace="Lys" /replace="Leu" /replace="Met" /replace="Gln" /replace="Pro" /replace="Arg" /replace="Ser" /replace="Thr" /replace="Val" /replace="Trp" /replace="Tyr"
  VARIANT (6)..(6): /replace="Ala" /replace="Cys" /replace="Asp" /replace="Trp" /replace="Phe" /replace="Gly" /replace="His" /replace="Ile" /replace="Lys" /replace="Leu" /replace="Met" /replace="Asn" /replace="Pro" /replace="Gln" /replace="Arg" /replace="Ser" /replace="Thr" /replace="Val" /replace="Tyr"
KNRWHE

SEQ ID NO: 33 - protein, 5 aa, Artificial Sequence
  peptide
  VARIANT (1)..(1): /replace="Ala" /replace="Cys" /replace="Asp" /replace="Glu" /replace="Phe" /replace="Gly" /replace="His" /replace="Ile" /replace="Leu" /replace="Met" /replace="Asn" /replace="Pro" /replace="Gln" /replace="Arg" /replace="Ser" /replace="Thr" /replace="Val" /replace="Trp" /replace="Tyr"
  VARIANT (5)..(5): /replace="Ala" /replace="Cys" /replace="Asp" /replace="Gln" /replace="Phe" /replace="Gly" /replace="His" /replace="Ile" /replace="Lys" /replace="Leu" /replace="Met" /replace="Asn" /replace="Pro" /replace="Arg" /replace="Ser" /replace="Thr" /replace="Val" /replace="Trp" /replace="Tyr"
KRWHE

SEQ ID NO: 34 - protein, 5 aa, Artificial Sequence
  peptide
KRWHE

SEQ ID NO: 35 - protein, 6 aa, Artificial Sequence
  peptide
KNRWHE

SEQ ID NO: 36 - protein, 7 aa, Artificial Sequence
  peptide
KGNRWHE

SEQ ID NO: 37 - protein, 5 aa, Artificial Sequence
  peptide
NAAAE

SEQ ID NO: 38 - protein, 13 aa, Artificial Sequence
  peptide
  VARIANT (1)..(1): /replace="Ala" /replace="Cys" /replace="Asp" /replace="Glu" /replace="Phe" /replace="Gly" /replace="His" /replace="Ile" /replace="Leu" /replace="Met" /replace="Asn" /replace="Pro" /replace="Gln" /replace="Arg" /replace="Ser" /replace="Thr" /replace="Val" /replace="Trp" /replace="Tyr"
  VARIANT (2)..(2): /replace="Ala" /replace="Cys" /replace="Asp" /replace="Phe" /replace="Gly" /replace="His" /replace="Ile" /replace="Lys" /replace="Leu" /replace="Met" /replace="Asn" /replace="Pro" /replace="Gln" /replace="Arg" /replace="Ser" /replace="Thr" /replace="Val" /replace="Trp" /replace="Tyr"
  VARIANT (3)..(3): /replace="Ala" /replace="Cys" /replace="Asp" /replace="Glu" /replace="Phe" /replace="Gly" /replace="His" /replace="Ile" /replace="Lys" /replace="Leu" /replace="Met" /replace="Asn" /replace="Pro" /replace="Arg" /replace="Ser" /replace="Thr" /replace="Val" /replace="Trp" /replace="Tyr"
  VARIANT (4)..(4): /replace="Ala" /replace="Cys" /replace="Asp" /replace="Glu" /replace="Phe" /replace="Gly" /replace="His" /replace="Ile" /replace="Lys" /replace="Leu" /replace="Met" /replace="Asn" /replace="Pro" /replace="Gln" /replace="Arg" /replace="Ser" /replace="Thr" /replace="Val" /replace="Tyr"
  VARIANT (5)..(5): /replace="Ala" /replace="Cys" /replace="Asp" /replace="Glu" /replace="Gly" /replace="His" /replace="Ile" /replace="Lys" /replace="Leu" /replace="Met" /replace="Asn" /replace="Pro" /replace="Gln" /replace="Arg" /replace="Ser" /replace="Thr" /replace="Val" /replace="Trp" /replace="Tyr"
  VARIANT (6)..(6): /replace="Ala" /replace="Cys" /replace="Asp" /replace="Glu" /replace="Phe" /replace="His" /replace="Ile" /replace="Lys" /replace="Leu" /replace="Met" /replace="Asn" /replace="Pro" /replace="Gln" /replace="Arg" /replace="Ser" /replace="Thr" /replace="Val" /replace="Trp" /replace="Tyr"
  VARIANT (7)..(7): /replace="Ala" /replace="Cys" /replace="Asp" /replace="Glu" /replace="Phe" /replace="Gly" /replace="His" /replace="Ile" /replace="Lys" /replace="Leu" /replace="Met" /replace="Pro" /replace="Gln" /replace="Arg" /replace="Ser" /replace="Thr" /replace="Val" /replace="Trp" /replace="Tyr"
  VARIANT (11)..(11): /replace="Ala" /replace="Cys" /replace="Asp" /replace="Phe" /replace="Gly" /replace="His" /replace="Ile" /replace="Lys" /replace="Leu" /replace="Met" /replace="Asn" /replace="Pro" /replace="Gln" /replace="Arg" /replace="Ser" /replace="Thr" /replace="Val" /replace="Trp" /replace="Tyr"
  VARIANT (12)..(12): /replace="Ala" /replace="Cys" /replace="Asp" /replace="Glu" /replace="Phe" /replace="His" /replace="Ile" /replace="Lys" /replace="Leu" /replace="Met" /replace="Asn" /replace="Pro" /replace="Gln" /replace="Arg" /replace="Ser" /replace="Thr" /replace="Val" /replace="Trp" /replace="Tyr"
  VARIANT (13)..(13): /replace="Ala" /replace="Cys" /replace="Asp" /replace="Glu" /replace="Phe" /replace="Gly" /replace="His" /replace="Ile" /replace="Lys" /replace="Leu" /replace="Met" /replace="Asn" /replace="Pro" /replace="Gln" /replace="Arg" /replace="Ser" /replace="Thr" /replace="Val" /replace="Trp"
KEQWFGNRWHEGY

SEQ ID NO: 39 - protein, 12 aa, Artificial Sequence
  peptide
  VARIANT (1)..(1): /replace="Ala" /replace="Cys" /replace="Asp" /replace="Glu" /replace="Phe" /replace="Gly" /replace="His" /replace="Ile" /replace="Leu" /replace="Met" /replace="Asn" /replace="Pro" /replace="Gln" /replace="Arg" /replace="Ser" /replace="Thr" /replace="Val" /replace="Trp" /replace="Tyr"
  VARIANT (2)..(2): /replace="Ala" /replace="Cys" /replace="Asp" /replace="Phe" /replace="Gly" /replace="His" /replace="Ile" /replace="Lys" /replace="Leu" /replace="Met" /replace="Asn" /replace="Pro" /replace="Gln" /replace="Arg" /replace="Ser" /replace="Thr" /replace="Val" /replace="Trp" /replace="Tyr"
  VARIANT (3)..(3): /replace="Ala" /replace="Cys" /replace="Asp" /replace="Glu" /replace="Phe" /replace="Gly" /replace="His" /replace="Ile" /replace="Lys" /replace="Leu" /replace="Met" /replace="Asn" /replace="Pro" /replace="Arg" /replace="Ser" /replace="Thr" /replace="Val" /replace="Trp" /replace="Tyr"
  VARIANT (4)..(4): /replace="Ala" /replace="Cys" /replace="Asp" /replace="Glu" /replace="Phe" /replace="Gly" /replace="His" /replace="Ile" /replace="Lys" /replace="Leu" /replace="Met" /replace="Asn" /replace="Pro" /replace="Gln" /replace="Arg" /replace="Ser" /replace="Thr" /replace="Val" /replace="Tyr"
  VARIANT (5)..(5): /replace="Ala" /replace="Cys" /replace="Asp" /replace="Glu" /replace="Gly" /replace="His" /replace="Ile" /replace="Lys" /replace="Leu" /replace="Met" /replace="Asn" /replace="Pro" /replace="Gln" /replace="Arg" /replace="Ser" /replace="Thr" /replace="Val" /replace="Trp" /replace="Tyr"
  VARIANT (6)..(6): /replace="Ala" /replace="Cys" /replace="Asp" /replace="Glu" /replace="Phe" /replace="His" /replace="Ile" /replace="Lys" /replace="Leu" /replace="Met" /replace="Asn" /replace="Pro" /replace="Gln" /replace="Arg" /replace="Ser" /replace="Thr" /replace="Val" /replace="Trp" /replace="Tyr"
  VARIANT (7)..(7): /replace="Ala" /replace="Cys" /replace="Asp" /replace="Glu" /replace="Phe" /replace="Gly" /replace="His" /replace="Ile" /replace="Lys" /replace="Leu" /replace="Met" /replace="Pro" /replace="Gln" /replace="Arg" /replace="Ser" /replace="Thr" /replace="Val" /replace="Trp" /replace="Tyr"
  VARIANT (11)..(11): /replace="Ala" /replace="Cys" /replace="Asp" /replace="Phe" /replace="Gly" /replace="His" /replace="Ile" /replace="Lys" /replace="Leu" /replace="Met" /replace="Asn" /replace="Pro" /replace="Gln" /replace="Arg" /replace="Ser" /replace="Thr" /replace="Val" /replace="Trp" /replace="Tyr"
  VARIANT (12)..(12): /replace="Ala" /replace="Cys" /replace="Asp" /replace="Glu" /replace="Phe" /replace="His" /replace="Ile" /replace="Lys" /replace="Leu" /replace="Met" /replace="Asn" /replace="Pro" /replace="Gln" /replace="Arg" /replace="Ser" /replace="Thr" /replace="Val" /replace="Trp" /replace="Tyr"
KEQWFGNRWHEG

SEQ ID NO: 40 - protein, 11 aa, Artificial Sequence
  peptide
  VARIANT (1)..(1): /replace="Ala" /replace="Cys" /replace="Asp" /replace="Glu" /replace="Phe" /replace="Gly" /replace="His" /replace="Ile" /replace="Leu" /replace="Met" /replace="Asn" /replace="Pro" /replace="Gln" /replace="Arg" /replace="Ser" /replace="Thr" /replace="Val" /replace="Trp" /replace="Tyr"
  VARIANT (2)..(2): /replace="Ala" /replace="Cys" /replace="Asp" /replace="Phe" /replace="Gly" /replace="His" /replace="Ile" /replace="Lys" /replace="Leu" /replace="Met" /replace="Asn" /replace="Pro" /replace="Gln" /replace="Arg" /replace="Ser" /replace="Thr" /replace="Val" /replace="Trp" /replace="Tyr"
  VARIANT (3)..(3): /replace="Ala" /replace="Cys" /replace="Asp" /replace="Glu" /replace="Phe" /replace="Gly" /replace="His" /replace="Ile" /replace="Lys" /replace="Leu" /replace="Met" /replace="Asn" /replace="Pro" /replace="Arg" /replace="Ser" /replace="Thr" /replace="Val" /replace="Trp" /replace="Tyr"
  VARIANT (4)..(4): /replace="Ala" /replace="Cys" /replace="Asp" /replace="Glu" /replace="Phe" /replace="Gly" /replace="His" /replace="Ile" /replace="Lys" /replace="Leu" /replace="Met" /replace="Asn" /replace="Pro" /replace="Gln" /replace="Arg" /replace="Ser" /replace="Thr" /replace="Val" /replace="Tyr"
  VARIANT (5)..(5): /replace="Ala" /replace="Cys" /replace="Asp" /replace="Glu" /replace="Gly" /replace="His" /replace="Ile" /replace="Lys" /replace="Leu" /replace="Met" /replace="Asn" /replace="Pro" /replace="Gln" /replace="Arg" /replace="Ser" /replace="Thr" /replace="Val" /replace="Trp" /replace="Tyr"
  VARIANT (6)..(6): /replace="Ala" /replace="Cys" /replace="Asp" /replace="Glu" /replace="Phe" /replace="His" /replace="Ile" /replace="Lys" /replace="Leu" /replace="Met" /replace="Asn" /replace="Pro" /replace="Gln" /replace="Arg" /replace="Ser" /replace="Thr" /replace="Val" /replace="Trp" /replace="Tyr"
  VARIANT (7)..(7): /replace="Ala" /replace="Cys" /replace="Asp" /replace="Glu" /replace="Phe" /replace="Gly" /replace="His" /replace="Ile" /replace="Lys" /replace="Leu" /replace="Met" /replace="Pro" /replace="Gln" /replace="Arg" /replace="Ser" /replace="Thr" /replace="Val" /replace="Trp" /replace="Tyr"
  VARIANT (11)..(11): /replace="Ala" /replace="Cys" /replace="Asp" /replace="Phe" /replace="Gly" /replace="His" /replace="Ile" /replace="Lys" /replace="Leu" /replace="Met" /replace="Asn" /replace="Pro" /replace="Gln" /replace="Arg" /replace="Ser" /replace="Thr" /replace="Val" /replace="Trp" /replace="Tyr"
KEQWFGNRWHE